European Patent Application EP 4 653 534 A1, published November 26, 2025. Title: MICROORGANISM FOR PRODUCING L-TRYPTOPHAN AND METHOD FOR PRODUCING L-TRYPTOPHAN USING SAME. Applicant: CJ CHEILJEDANG CORPORATION. Application KR. The sequence listing filed with the application follows.

SEQUENCE LISTING (32 sequences)

SEQ ID NO: 1 - protein, 891 aa, unidentified
MTKWVYSFGDGLNEGRADMRNLLGGKGANLAEMAANGLPVPPGFTITTEVCSAFYENGRKYPDELKAQVDAALQRVEQSMGLRFGDPEAPLLVSVRSGARVSMPGMMDTVLNLGLNDQTVEGLARSSGDARFAWDSYRRFIQMYGSVVMGVPHHHFEDVLEQFKRANNVEDDTAITAGQWRAIVVDYTHIITTHTGTDFPTNPQDQLWGAIGAVFGSWMNPRANTYRKLHEIPASWGTAVNVQSMVFGNMGDDCATGVCFTRDPSTGENIFYGEYLINAQGEDVVAGIRTPQPMACARAEAGQHPMETTLPQAYAELLRVRSILETHYKDMQDIEFTVQRNVLYILQTRNGKRTAAAALKIAIDMAREGLITQEEAIQRVPAASLDQLLHPTLDPRAERVQLTRGLPASPGAAAGAVVFTAEECEARAAKGEDVILVRIETSPEDVHGMHAARGVLTTRGGMTSHAAVVARGMGRVCVAGAGGIHVDYAAGSLSVGSHTVKEGEWITLDGGTGAVYLGRVPTIEPVLSDDFNTLMGWADGVRRLGVRANAETPDDARTARRFGAEGIGLARTEHMFFGPDRIGFVRQMIIADEESVRQKAIAALLPFQREDFASLFRIMAGLPVTVRLLDPPLHEFLPHEAAEMAEVAQALGRSVEDVRARCAALAETNPMLGHRGCRLGLTSPEIYAMQVRALIQAAVLVEKELGRPIHPEIMIPLVATKAELATTRRAAEDEIARVLKEEGTNLSYSIGTMIELPRAAIQADQIAEYADFFSFGTNDLTQTTFGLSRDDAGSFLPYYVDQGLLPRDPFVSIDRDGVGALVRLGVERGRQTSADLKLGICGEHGGDPDSIAFFDEVGLDYVSCSPFRVPVARLAAAQAALATRQKAASPA

SEQ ID NO: 2 - DNA, 2676 bp, unidentified
  source 1..2676: mol_type = genomic DNA
atgaccaaatgggtttacagcttcggggatggcctgaatgaaggtcgcgcggatatgcgcaaccttcttggtggcaagggcgccaatctggcggaaatggcggcgaacggcctgccggtgccgccgggctttaccattacgacggaagtctgttcggctttctatgaaaacggccgtaaatatcccgatgaactgaaggcgcaggtcgatgccgcccttcagcgtgtcgagcagtccatgggcctgcgctttggtgaccccgaagccccgctgctggtctcggtgcgttcgggtgcgcgggtgtccatgccgggcatgatggataccgtgctcaacctgggcctgaatgaccagacggtggaagggcttgcccgttcctcgggcgatgcgcgcttcgcgtgggacagctaccgccgcttcatccagatgtacggctcggtcgtgatgggcgtgccccatcaccatttcgaggacgtgctggagcagttcaagcgcgccaacaatgtggaggacgacaccgccatcaccgccgggcagtggcgcgcgatcgtggtggactacacccacatcatcacaacccataccggcaccgatttccccaccaatccgcaggaccagctgtggggcgccatcggcgccgtgttcggttcgtggatgaacccgcgcgccaacacctatcgcaagctgcacgagatcccggcttcgtgggggacggcggtcaacgtgcagtccatggtgttcggcaacatgggcgatgactgcgcgaccggcgtgtgcttcacccgcgatccctcgacgggcgagaacatcttctacggtgaatacctgatcaacgcgcagggcgaggacgtggtggcgggcatccgcacgccgcagcccatggcctgcgcccgcgccgaggccggccagcacccgatggaaaccaccctgccgcaggcttacgccgaactgctgcgcgtgcgctccatactggaaacccattacaaggacatgcaggacatcgaattcacggtccagcgcaacgtcctgtacattctccagacccgcaacggcaagcgcacggccgccgccgcgctgaagatcgccatcgacatggcgcgtgaagggctgatcacgcaggaagaggccatccagcgcgtgcctgcggcctcccttgaccagcttctgcaccccacactggaccccagggccgagcgtgtgcagctgacccgtggtcttccggcctcgcccggtgcggccgccggtgccgtcgtgttcacggcggaggaatgcgaggcccgcgcggcgaaaggggaggatgtgatccttgtgcggatcgagacctcgcccgaggacgtgcatggcatgcacgccgcccggggcgtgctgaccacccgtggcggcatgacgtcgcacgccgccgtggtggcgcgtggcatgggccgcgtatgcgtggccggtgccggcggcatccatgtcgattacgcggcaggcagcctgagtgtcggctcccataccgtgaaggaaggcgagtggatcacgctcgatggcgggacgggcgcggtctatctggggcgcgtgccgaccatcgaacccgtgctgtcggatgatttcaacacgctcatggggtgggcggacggcgtgcgccgcctgggcgtgcgcgccaatgccgaaacgccggatgacgcgcgcaccgcgcgccgcttcggcgcggaggggattggcctggcgcgtaccgagcacatgttcttcggccctgaccgcatcggctttgtccgccagatgatcattgccgatgaggagagcgtgcgccagaaggccatcgccgccctgctgccgttccagcgcgaggattttgccagcctgttccgcatcatggccgggctgccggtcacggtgcgcctgctggacccgccgctgcacgagttcctgccgcatgaggcggccgagatggccgaggtggcacaggcgctgggcaggagcgtggaggacgtgcgcgcgcgttgcgccgctctggcggaaaccaacccgatgctgggccaccgtggctgccgccttggcctgaccagtccggaaatctatgccatgcaggtccgtgcgctgatccaggcggcggtactggtggaaaaggaactgggcaggcccatccaccccgagatcatgatcccgctggtggcgacaaaggccgaactggccaccacccgccgtgcggccgaggacgagatcgcgcgtgtgctgaaggaggaggggacgaatctcagctactccatcggcaccatgatcgaactgccccgtgccgccatccaggcggaccagatcgcggaatatgccgatttcttctcgttcggcaccaacgacctgacccagaccaccttcggcctgtcgcgtgatgatgcggggtccttcctgccctattacgttgaccaggggctgctgccgcgtgatccgttcgtgtcgatcgaccgcgatggcgtgggggcgcttgtccgccttggggtggaacgtggccgtcagaccagcgcggacctgaagctgggcatctgcggcgaacatggtggcgacccggattccatcgcattctttgatgaagtcgggctggactatgtctcgtgctcgcccttccgcgtgccggtggcacgtcttgccgcggcacaggccgcgctggccacgcgccagaaggccgccagcccggcctga

SEQ ID NO: 3 - protein, 873 aa, Acetobacter pasteurianus
MRNLLGGKGANLAEMANIGLPVPPGFTITTEVCTAFYENGRKYPAELESQLEEAMGLVEKAMGLRFGDANAPLLVSVRSGARVSMPGMMDTVLNLGLNDSTVEGLVKSSGDARFAWDSYRRFIQMYGSVVLGVAHHRFEDLLEQIKRAIGKEDDTSLTAEEWQEVVKGYKQIVLQETGTAFPESPKEQLWGAIGAVFGSWMNPRANTYRKLHDIPASWGTAVNVQSMVFGNMGDDCATGVCFTRDPSTGENIFYGEYLINAQGEDVVAGIRTPQPMAASRAAEGQVPMEKALPNAYQELLKVRDLLERHYRDMQDIEFTVQANKLYLLQTRSGKRTAAAALRIAIDMAKENLITQEEAVNRVPPASLDQLLHPVLDPKAERQLLTRGLPASPGAATGVIAFSAEDVEDRAAKGEDVILVRVETSPEDVHGMHAARGVLTTRGGMTSHAAVVARGMGRVCVAGAGSIAVDYKAQTMKVDGHTLKAGDWLTLDGGTGAVYKGRVPTIPPTLSGDFATLMGWADSIRRLGVRANAETPEDAATARRFGAEGIGLCRTEHMFFGPDRIGHVRQMIMADDKATRAKAINALLPFQRSDFTELFRIMAGLPVTIRLLDPPLHEFLPHGEAELEEVAKALGQDVETLRARRSALSEANPMLGHRGCRLGITYPEIYAMQVRAIAEAALNIAKETGKPVTPEIMIPLIGTKAELDLVRKTCETAIADVLSERKAELSYKIGTMIELPRAAITADQIAQSADFFSFGTNDLTQTTLGLSRDDAGSFLPEYVEKGLLPQDPFVSIDREGVGALVRMGVEKGRATKPDIKLGICGEHGGDPLSISFFEEVGLDYVSCSPFRVPVARLAAAQAALAAKNNKAVKA

SEQ ID NO: 4 - DNA, 2622 bp, Acetobacter pasteurianus
  source 1..2622: mol_type = genomic DNA
atgcgcaatctcctcggcggtaagggagccaatctggcagaaatggccaatatcggcctgcccgtcccccccggatttaccattaccactgaagtctgcacggcgttctacgaaaacggacggaaatacccggctgagctggaatcccagcttgaagaagccatgggtctggttgaaaaagccatgggcctgcgctttggcgatgccaatgcccccctgcttgtttctgtccgttctggcgcacgtgtttccatgcccggcatgatggatacagttctcaacctagggctgaatgacagcactgttgaaggacttgtaaaatcatccggtgatgcccggtttgcatgggatagctaccgccgcttcattcagatgtacggctctgttgtgctaggtgttgcccaccaccgctttgaagatctgcttgagcagatcaagcgtgccatcggcaaggaagacgatacgtctctgaccgctgaagaatggcaggaagtcgttaaaggctacaaacagattgttctgcaggaaaccggcaccgcctttcctgaaagcccgaaagaacagctttggggcgccattggagccgtgtttggttcatggatgaacccacgcgccaacacttaccgcaagctgcacgatattccggcaagctggggcacggctgttaacgtgcagtccatggtgttcggcaacatgggtgatgattgcgccaccggcgtctgcttcacgcgtgatccttccaccggtgaaaacattttctacggtgaatacctgatcaacgcgcagggtgaagacgttgtggccggtatccgcacaccgcagcccatggcggcatctcgtgcggctgaaggccaggtgcctatggaaaaggccctacccaacgcgtatcaggaactgctgaaagtgcgcgatctgctggaacgccactaccgcgatatgcaggacattgagtttacggtgcaggccaacaagctgtacctgctccagactcgttcgggcaaacgcacagccgcagccgccctgcgcattgccattgatatggccaaggaaaacctgatcacgcaggaagaagccgttaaccgcgtgccgcctgcatctcttgatcagctcctgcaccctgtgctggaccccaaggcagaacgtcagcttcttacacgtggccttcccgcttctccgggggctgcaacaggcgtgatcgcgttctcagctgaagatgtggaagaccgcgctgccaagggtgaagatgttattctggtgcgtgttgaaacctccccggaagacgtacacggcatgcacgctgcccgcggtgtgctgacaactcgtggcggcatgacatcccatgccgctgtggtggcccgtggcatgggccgcgtgtgcgtggccggtgctggcagcattgccgtggattacaaagcccagaccatgaaagtggacggtcacacactcaaagcgggtgactggctgacactggatggtggcacgggcgctgtttacaaaggccgtgttcccaccattccgccaacactctctggtgactttgcaacccttatggggtgggcagattccatccgtcgccttggtgtgcgcgctaatgctgaaacgccagaagatgcggcaacagcccgccgctttggtgcagaaggtattggcctgtgccgcacagagcacatgttcttcggcccggatcggattggccatgtgcgccagatgatcatggcggatgacaaagccacacgcgccaaagctattaacgcgcttctacccttccagcggagtgactttacagaactgttccgcattatggcggggctgcctgttaccatccgtctgcttgatccaccgctgcacgaattcctgccgcatggtgaagcagagctggaagaagttgccaaagcacttgggcaggatgtcgaaaccctgcgtgctcgtcgctctgcgctatctgaagccaacccaatgctgggccaccgtggctgccgtctgggtattacatacccggaaatctacgccatgcaggtgcgtgccattgcagaagcggctcttaatatcgccaaggaaacaggcaagcctgttaccccagaaatcatgattccgctaattggcacaaaagcagagctggatctggtgcgtaaaacctgtgaaaccgccattgctgatgttctttctgaacgcaaagctgagctgtcttacaaaatcggcaccatgattgagctgccacgcgcagccattacggcagaccagattgcacagagcgcagacttcttctccttcggcacaaacgatctgacacagaccacccttggactttcccgcgatgatgctggctccttcttgccagaatacgtggaaaaagggctgctgccgcaggacccgtttgtttcgatcgaccgtgaaggcgttggcgcactggtgcgtatgggtgttgaaaaaggccgtgcaaccaagcctgacatcaaactgggtatctgtggtgaacacgggggcgatccgctttccatctccttctttgaagaagttgggctggattacgtctcctgctcccccttccgggtgcccgttgccagattggccgcagcacaggccgcactggctgctaaaaacaacaaggccgtaaaagcctga

SEQ ID NO: 5 - protein, 802 aa, Methanosarcina acetivorans
MPGDKNKYIRWFEETTIEDVPLVGGKNASLGEMYRELTSKGVRIPNGFSVTSEAYWHMLKAGGILEKLKKTMEGLDTSNVSDLAKRGKAARDLILGAGLPDDLWEEIKASYDRLCEQYGEDTDVAVRSSATAEDLPTASFAGQQETYLNIRGYPGLRDACIRCFASLFTDRAISYRVTNNFDHFKVALSIGIMKMVRSDLASSGVIFTLDTETGFRDVVFITGAYGLGENVVQGQVNPDEFYVFKPTFREGHKPIIQKKLGSKEIKMIYGRGDSKVLTRNVEVPEAERLRFCINDEEVLKLAGYAIDIEEHYSNKYGESRPMDIEWAKDGITGELFIVQARPETVQSQRAKDVLETYVLEKKSEVLAKGRSVGDKIASGKAHVIPDVSDLPSFRPGEILIADTTTPDWEPVMKTAAAIVTNKGGRTCHAAIVSRELGIPAVVGAGNATEVLETGREITVSCAEGEDGFVYAGLLPFHKDTMSLKDLKRPGTEIMMNLGNPESAFAYSMIPNDGIGLARLEFIITSYIKVHPMALVHPEKVKAQGEIQEIEGLTRGYEKKEDYFVDQLARGVGMITAAFYPKPVVVRMSDFKTNEYASLVGGSYFEMDENNPMIGFRGASRYFDERYREGFALECRAMKKVRDEMGLTNLILMIPFCRTVEEAEKVIAEMEKNDLRRGENGLQVYVMCEIPNNVLLVDEFSEFFDGFSIGSNDLTQLTLGVDRDSELLAAEFDERDPGVMKIMSMAVQGAKRNKRHSGICGQAPSDFPEIAEFLVKEGINSISLNPDSVMKITLKVLETEKEL

SEQ ID NO: 6 - DNA, 2409 bp, Methanosarcina acetivorans
  source 1..2409: mol_type = genomic DNA
atgcctggagataaaaacaaatacatccgctggtttgaagagaccacgatcgaggacgtcccgctggttggcggaaagaatgcttcccttggggagatgtacagggaacttacttcaaaaggtgtgaggatcccgaatggcttttcagttacttccgaggcttactggcacatgctgaaggcaggaggaattctcgaaaaacttaaaaagacaatggaagggcttgatacctcaaatgtgtcagaccttgcaaagaggggaaaggccgcaagagacctgattcttggtgcgggacttccggatgatctctgggaggagatcaaagcttcttacgatcgactctgcgagcagtacggagaggacacggatgtggctgtcaggagttcggcaacggccgaggatctgcctaccgcttcttttgcggggcagcaggagacttacctcaatattcggggatatccaggacttcgggacgcctgtatacgctgttttgcttctctttttacggatagggccatttcctaccgcgtaaccaacaatttcgaccactttaaggtagccctttccataggaatcatgaagatggtcagatcggatctggcttcaagcggtgtgatttttactcttgacacggaaacgggtttcagggatgttgttttcattaccggagcatacgggctcggcgagaatgtcgttcagggccaggtaaaccctgatgagttctatgtcttcaagcccactttcagggaagggcataagccgattatccagaagaagctggggagcaaagaaatcaagatgatctacggcaggggagactcaaaagtcctcacaaggaatgtggaggtccctgaggctgaaaggctgcgcttctgtatcaatgacgaagaagtgctcaaacttgccgggtatgcgatcgatattgaggaacattattctaacaagtacggggaatccaggcccatggatatcgagtgggcaaaggacggtataacaggcgaactcttcatagtgcaggcaaggcccgaaaccgtccagtcccagagagcaaaggatgtgctggaaacttatgtccttgaaaagaagtccgaagtccttgcaaaaggcaggagcgtgggagataagatcgcatccggaaaagcccacgtgatccccgatgtttccgacctgccttctttcaggcccggggaaatcctgatcgcggatacgaccactcctgactgggaaccggttatgaaaaccgcagctgcgattgtcaccaacaagggaggcaggacctgtcatgcggcgattgtcagcagggaactcggaatccctgcggttgtcggggctggaaatgctaccgaagtccttgagacaggcagggaaattaccgtgagctgtgccgaaggcgaagacgggtttgtatatgcagggctcctccccttccataaagataccatgagcctgaaagacctgaaacgcccagggaccgagattatgatgaaccttggaaaccctgaaagtgcttttgcgtattccatgattcctaacgacgggatcgggcttgcaaggctcgagtttattatcacaagctacatcaaagtccatcccatggctcttgtgcaccctgaaaaagtcaaggctcagggggaaatccaagagatcgaagggctaacgcggggctatgagaaaaaggaagattattttgtcgatcagcttgccagaggcgtcggaatgattactgcggctttttacccaaagccggttgtggtcaggatgagcgatttcaagaccaatgagtacgcaagccttgtagggggcagctactttgaaatggacgaaaacaaccccatgataggattcaggggagcttcccgttactttgatgaacggtacagggaaggttttgcccttgagtgcagagctatgaaaaaagtcagggacgaaatggggcttacaaatcttattcttatgattcccttctgccggaccgttgaggaagcggagaaagtcatcgccgagatggagaaaaacgatctcaggcgcggagaaaacgggcttcaggtctatgttatgtgcgaaatccccaataacgtcctgcttgtcgacgaattcagtgaattctttgacggtttttccattggctcaaatgacctgacccagctgaccctgggggttgaccgcgactctgaactccttgccgcggaattcgatgagcgggatccgggggtcatgaaaatcatgtcaatggcagtgcagggggcaaagcgaaataaaaggcacagcgggatatgcgggcaggctccgagtgatttcccggagattgcagaattcctggtaaaagaggggatcaattcgatttcccttaatccggactctgttatgaaaatcacccttaaggttctcgaaactgaaaaggagctctga

SEQ ID NO: 7 - protein, 792 aa, Escherichia coli
MSNNGSSPLVLWYNQLGMNDVDRVGGKNASLGEMITNLSGMGVSVPNGFATTADAFNQFLDQSGVNQRIYELLDKTDIDDVTQLAKAGAQIRQWIIDTPFQPELENAIREAYAQLSADDENASFAVRSSATAEDMPDASFAGQQETFLNVQGFDAVLVAVKHVFASLFNDRAISYRVHQGYDHRGVALSAGVQRMVRSDLASSGVMFSIDTESGFDQVVFITSAWGLGEMVVQGAVNPDEFYVHKPTLAANRPAIVRRTMGSKKIRMVYAPTQEHGKQVKIEDVPQEQRDIFSLTNEEVQELAKQAVQIEKHYGRPMDIEWAKDGHTGKLFIVQARPETVRSRGQVMERYTLHSQGKIIAEGRAIGHRIGAGPVKVIHDISEMNRIEPGDVLVTDMTDPDWEPIMKKASAIVTNRGGRTCHAAIIARELGIPAVVGCGDATERMKDGENVTVSCAEGDTGYVYAELLEFSVKSSSVETMPDLPLKVMMNVGNPDRAFDFACLPNEGVGLARLEFIINRMIGVHPRALLEFDDQEPQLQNEIREMMKGFDSPREFYVGRLTEGIATLGAAFYPKRVIVRLSDFKSNEYANLVGGERYEPDEENPMLGFRGAGRYVSDSFRDCFALECEAVKRVRNDMGLTNVEIMIPFVRTVDQAKAVVEELARQGLKRGENGLKIIMMCEIPSNALLAEQFLEYFDGFSIGSNDMTQLALGLDRDSGVVSELFDERNDAVKALLSMAIRAAKKQGKYVGICGQGPSDHEDFAAWLMEEGIDSLSLNPDTVVQTWLSLAELKK

SEQ ID NO: 8 - DNA, 2379 bp, Escherichia coli
  source 1..2379: mol_type = genomic DNA
atgtccaacaatggctcgtcaccgctggtgctttggtataaccaactcggcatgaatgatgtagacagggttgggggcaaaaatgcctccctgggtgaaatgattactaatctttccggaatgggtgtttccgttccgaatggtttcgccacaaccgccgacgcgtttaaccagtttctggaccaaagcggcgtaaaccagcgcatttatgaactgctggataaaacggatattgacgatgttactcagcttgcgaaagcgggcgcgcaaatccgccagtggattatcgacactcccttccagcctgagctggaaaacgccatccgcgaagcctatgcacagctttccgccgatgacgaaaacgcctcttttgcggtgcgctcctccgccaccgcagaagatatgccggacgcttcttttgccggtcagcaggaaaccttcctcaacgttcagggttttgacgccgttctcgtggcagtgaaacatgtatttgcttctctgtttaacgatcgcgccatctcttatcgtgtgcaccagggttacgatcaccgtggtgtggcgctctccgccggtgttcaacggatggtgcgctctgacctcgcatcatctggcgtgatgttctccattgataccgaatccggctttgaccaggtggtgtttatcacttccgcatggggccttggtgagatggtcgtgcagggtgcggttaacccggatgagttttacgtgcataaaccgacactggcggcgaatcgcccggctatcgtgcgccgcaccatggggtcgaaaaaaatccgcatggtttacgcgccgacccaggagcacggcaagcaggttaaaatcgaagacgtaccgcaggaacagcgtgacatcttctcgctgaccaacgaagaagtgcaggaactggcaaaacaggccgtacaaattgagaaacactacggtcgcccgatggatattgagtgggcgaaagatggccacaccggtaaactgttcattgtgcaggcgcgtccggaaaccgtgcgctcacgcggtcaggtcatggagcgttatacgctgcattcacagggtaagattatcgccgaaggccgtgctatcggtcatcgcatcggtgcgggtccggtgaaagtcatccatgacatcagcgaaatgaaccgcatcgaacctggcgacgtgctggttactgacatgaccgacccggactgggaaccgatcatgaagaaagcatctgccatcgtcaccaaccgtggcggtcgtacctgtcacgcggcgatcatcgctcgtgaactgggcattccggcggtagtgggctgtggagatgcaacagaacggatgaaagacggtgagaacgtcactgtttcttgtgccgaaggtgataccggttacgtctatgcggagttgctggaatttagcgtgaaaagctccagcgtagaaacgatgccggatctgccgttgaaagtgatgatgaacgtcggtaacccggaccgtgctttcgacttcgcctgcctaccgaacgaaggcgtgggccttgcgcgtctggaatttatcatcaaccgtatgattggcgtccacccacgcgcactgcttgagtttgacgatcaggaaccgcagttgcaaaacgaaatccgcgagatgatgaaaggttttgattctccgcgtgaattttacgttggtcgtctgactgaagggatcgcgacgctgggtgccgcgttttatccgaagcgcgtcattgtccgtctctctgattttaaatcgaacgaatatgccaacctggtcggtggtgagcgttacgagccagatgaagagaacccgatgctcggcttccgtggcgcgggccgctatgtttccgacagcttccgcgactgtttcgcgctggagtgtgaagcagtgaaacgtgtgcgcaacgacatgggactgaccaacgttgagatcatgatcccgttcgtgcgtaccgtagatcaggcgaaagcggtggttgaagaactggcgcgtcaggggctgaaacgtggcgagaacgggctgaaaatcatcatgatgtgtgaaatcccgtccaacgccttgctggccgagcagttcctcgaatatttcgacggcttctcaattggctcaaacgatatgacgcagctggcgctcggtctggaccgtgactccggcgtggtgtctgaattgttcgatgagcgcaacgatgcggtgaaagcactgctgtcgatggctatccgtgccgcgaagaaacagggcaaatatgtcgggatttgcggtcagggtccgtccgaccacgaagactttgccgcatggttgatggaagaggggatcgatagcctgtctctgaacccggacaccgtggtgcaaacctggttaagcctggctgaactgaagaaataa

SEQ ID NO: 9 - protein, 364 aa, Corynebacterium glutamicum
MTNSLNIPFVQRFDEGLDPVLEVLGGKGASLVTMTDAGMPVPPGFVVTTASFDEFIREAGVAEHIDKFLNDLDAEDIKEVDRVSAIIRDELCSLEVPENARFAVHQAYRDLMERCGGDIPVAVRSSATAEDLPDASFAGQQDTYLWQVGLSAVTEHIRKCWASLFTSRAIIYRLKNNIPNEGLSMAVVVQKMVNSRVAGVAITMNPSNGDRSKITIDSSWGVGEMVVSGEVTPDNILLDKITLQVVSEHIGSKHAELIPDATSGSLVEKPVDEERANRRSLTDEEMLAVAQMAKRAEKHYKCPQDIEWALDADLPDGENLLLLQSRPETIHSNGVKKETPTPQAAKTTGTFDFSSITVAMTGTK

SEQ ID NO: 10 - DNA, 1095 bp, Corynebacterium glutamicum
  source 1..1095: mol_type = genomic DNA
atgaccaacagtttgaacatcccgtttgtccagcgctttgatgaaggcctggatcctgttctagaagtactcggtggcaagggcgcttcactagtcaccatgaccgatgctggaatgcccgttccgcctggatttgtggtcactactgccagctttgatgaattcatccgtgaagcaggcgttgctgaacacatcgataaattccttaacgatctcgatgcagaagatattaaggaagtggatcgagtttctgcgatcatccgcgatgagctgtgcagcctcgaagttccagagaacgctcgtttcgcagtgcaccaggcttatcgcgatctcatggaacgatgcggtggcgacatcccggttgctgtccggtcatcggccactgccgaagatctgcccgatgcttccttcgcagggcaacaggacacctatctgtggcaagtcggtttgagcgctgtcactgaacacatccgtaaatgctgggcttcgctgttcacttcccgtgccattatctaccgtctgaaaaacaacatccccaatgagggcctctccatggcggtagttgttcaaaaaatggtcaactctcgtgtcgcaggcgtggcaatcactatgaatccttccaacggcgaccgctcgaagatcaccatcgattcctcatggggtgttggtgaaatggtggtctcaggtgaagtgacaccagacaatatcttgctggacaagatcacgctgcaggttgtctccgaacacattggaagcaaacacgctgaactcatccccgatgccaccagtggaagcctcgtggaaaagcccgttgatgaagaacgcgcaaaccgccgcagtctgactgatgaggaaatgctcgctgtggcacaaatggctaagcgtgcagaaaaacactacaagtgcccacaagatatcgaatgggcgctggacgctgatctgccagatggagaaaaccttctgttattgcaatcccgtccggaaaccatccactccaacggtgtgaagaaggaaaccccaactccgcaagctgccaaaaccaccggcaccttcgatttcagctcaatcaccgtcgcaatgaccggcacgaagtaa

SEQ ID NO: 11 - DNA, 36 bp, synthetic construct
  source 1..36: mol_type = other DNA
aattcgagctcggtacccgatggaactacgagactg

SEQ ID NO: 12 - DNA, 41 bp, synthetic construct
  source 1..41: mol_type = other DNA
tgacaatcaccgcatccagtactggatattcgagacagctt

SEQ ID NO: 13 - DNA, 40 bp, synthetic construct
  source 1..40: mol_type = other DNA
gctgtctcgaatatccagtactggatgcggtgattgtcag

SEQ ID NO: 14 - DNA, 39 bp, synthetic construct
  source 1..39: mol_type = other DNA
ggtcgactctagaggatcccctaaccacgacgactgcaa

SEQ ID NO: 15 - DNA, 36 bp, synthetic construct
  source 1..36: mol_type = other DNA
cgaaaggaaacactcatgaccaaatgggtttacagc

SEQ ID NO: 16 - DNA, 31 bp, synthetic construct
  source 1..31: mol_type = other DNA
aatcaccgcatccagttcaggccgggctggc

SEQ ID NO: 17 - DNA, 35 bp, synthetic construct
  source 1..35: mol_type = other DNA
tctcgaatatccagtagaaacatcccagcgctact

SEQ ID NO: 18 - DNA, 35 bp, synthetic construct
  source 1..35: mol_type = other DNA
aacccatttggtcatgagtgtttcctttcgttggg

SEQ ID NO: 19 - DNA, 20 bp, synthetic construct
  source 1..20: mol_type = other DNA
aacaacaccacatctacatc

SEQ ID NO: 20 - DNA, 18 bp, synthetic construct
  source 1..18: mol_type = other DNA
cagccttttccagcacca

SEQ ID NO: 21 - DNA, 33 bp, synthetic construct
  source 1..33: mol_type = other DNA
cgaaaggaaacactcatgcgcaatctcctcggc

SEQ ID NO: 22 - DNA, 41 bp, synthetic construct
  source 1..41: mol_type = other DNA
gctgacaatcaccgcatccagttcaggcttttacggccttg

SEQ ID NO: 23 - DNA, 35 bp, synthetic construct
  source 1..35: mol_type = other DNA
gaggagattgcgcatgagtgtttcctttcgttggg

SEQ ID NO: 24 - DNA, 43 bp, synthetic construct
  source 1..43: mol_type = other DNA
acgaaaggaaacactcatgcctggagataaaaacaaatacatc

SEQ ID NO: 25 - DNA, 37 bp, synthetic construct
  source 1..37: mol_type = other DNA
aatcaccgcatccagttcagagctccttttcagtttc

SEQ ID NO: 26 - DNA, 35 bp, synthetic construct
  source 1..35: mol_type = other DNA
tttatctccaggcatgagtgtttcctttcgttggg

SEQ ID NO: 27 - DNA, 35 bp, synthetic construct
  source 1..35: mol_type = other DNA
aacgaaaggaaacactcatgtccaacaatggctcg

SEQ ID NO: 28 - DNA, 38 bp, synthetic construct
  source 1..38: mol_type = other DNA
aatcaccgcatccagtttatttcttcagttcagccagg

SEQ ID NO: 29 - DNA, 35 bp, synthetic construct
  source 1..35: mol_type = other DNA
gccattgttggacatgagtgtttcctttcgttggg

SEQ ID NO: 30 - DNA, 40 bp, synthetic construct
  source 1..40: mol_type = other DNA
caacgaaaggaaacactcatgaccaacagtttgaacatcc

SEQ ID NO: 31 - DNA, 38 bp, synthetic construct
  source 1..38: mol_type = other DNA
acaatcaccgcatccagtttacttcgtgccggtcattg

SEQ ID NO: 32 - DNA, 35 bp, synthetic construct
  source 1..35: mol_type = other DNA
caaactgttggtcatgagtgtttcctttcgttggg